European Patent Application EP 4 538 390 A2, published April 16, 2025. Title: METHODS AND COMPOSITIONS FOR ANALYZING NUCLEIC ACID. Applicant: CLARET BIOSCIENCE, LLC. Application EP. The sequence listing filed with the application follows.

SEQUENCE LISTING (41 sequences)

SEQ ID NO: 1 - DNA, 20 bp, synthetic construct
  misc_feature 1..20: note = Description of Artificial Sequence: Synthetic oligonucleotide
  source 1..20: mol_type = other DNA
tttttttttttttttttttt

SEQ ID NO: 2 - skipped

SEQ ID NO: 3 - DNA, 51 bp, synthetic construct
  misc_difference 51: note = a, c, t, g, unknown or other
  misc_feature 1..51: note = Description of Artificial Sequence: Synthetic oligonucleotide
  source 1..51: mol_type = other DNA
ccatactgtggtcgtcacctattaccccgcgtaaaggtaggctatgtcatn

SEQ ID NO: 4 - DNA, 52 bp, synthetic construct
  misc_difference 51..52: note = a, c, t, g, unknown or other
  misc_feature 1..52: note = Description of Artificial Sequence: Synthetic oligonucleotide
  source 1..52: mol_type = other DNA
gtgaattgttgatgtcctgggtgcctcgtcccaaaagctgtcctcacgacnn

SEQ ID NO: 5 - DNA, 53 bp, synthetic construct
  misc_difference 51..53: note = a, c, t, g, unknown or other
  misc_feature 1..53: note = Description of Artificial Sequence: Synthetic oligonucleotide
  source 1..53: mol_type = other DNA
gcttctcgaacccgcgatccggccgatccggcataatgggttgatttagannn

SEQ ID NO: 6 - DNA, 54 bp, synthetic construct
  misc_difference 51..54: note = a, c, t, g, unknown or other
  misc_feature 1..54: note = Description of Artificial Sequence: Synthetic oligonucleotide
  source 1..54: mol_type = other DNA
cgacacggatattccatcaagagacgggcctatggtccctgtgatgatgtnnnn

SEQ ID NO: 7 - DNA, 55 bp, synthetic construct
  misc_difference 51..55: note = a, c, t, g, unknown or other
  misc_feature 1..55: note = Description of Artificial Sequence: Synthetic oligonucleotide
  source 1..55: mol_type = other DNA
accttgtgtgttgctgaagcaaagccgcgtgaccgttttaaccagcgaacnnnnn

SEQ ID NO: 8 - DNA, 56 bp, synthetic construct
  misc_difference 51..56: note = a, c, t, g, unknown or other
  misc_feature 1..56: note = Description of Artificial Sequence: Synthetic oligonucleotide
  source 1..56: mol_type = other DNA
attttaccacgagttccttacgacggctgtgatgccacggtaggcaggtannnnnn

SEQ ID NO: 9 - DNA, 51 bp, synthetic construct
  misc_difference 1: note = a, c, t, g, unknown or other
  misc_feature 1..51: note = Description of Artificial Sequence: Synthetic oligonucleotide
  source 1..51: mol_type = other DNA
ncgctttacgggtcctgggccggggtgcgataccttgcagaaatcgaggcc

SEQ ID NO: 10 - DNA, 52 bp, synthetic construct
  misc_difference 1..2: note = a, c, t, g, unknown or other
  misc_feature 1..52: note = Description of Artificial Sequence: Synthetic oligonucleotide
  source 1..52: mol_type = other DNA
nnaggactctgccgtcgacgagttcgttaattcacggcatcacgtgcgtagt

SEQ ID NO: 11 - DNA, 53 bp, synthetic construct
  misc_difference 1..3: note = a, c, t, g, unknown or other
  misc_feature 1..53: note = Description of Artificial Sequence: Synthetic oligonucleotide
  source 1..53: mol_type = other DNA
nnnacctccgtcgcgctatgttctgttgcattcgaccttctccgttctgtggg

SEQ ID NO: 12 - DNA, 54 bp, synthetic construct
  misc_difference 1..4: note = a, c, t, g, unknown or other
  misc_feature 1..54: note = Description of Artificial Sequence: Synthetic oligonucleotide
  source 1..54: mol_type = other DNA
nnnnacaagaggagcatccgtattaccgcctatatcgcctacgtttagagcatt

SEQ ID NO: 13 - DNA, 55 bp, synthetic construct
  misc_difference 1..5: note = a, c, t, g, unknown or other
  misc_feature 1..55: note = Description of Artificial Sequence: Synthetic oligonucleotide
  source 1..55: mol_type = other DNA
nnnnngtaaatcccacacagctgtcggcttatatggtcattggacggcgtaatag

SEQ ID NO: 14 - DNA, 56 bp, synthetic construct
  misc_difference 1..6: note = a, c, t, g, unknown or other
  misc_feature 1..56: note = Description of Artificial Sequence: Synthetic oligonucleotide
  source 1..56: mol_type = other DNA
nnnnnnccagacagccatagaggttacaagcatagcaatttgcatcagttcgcaga

SEQ ID NO: 15 - DNA, 50 bp, synthetic construct
  misc_feature 1..50: note = Description of Artificial Sequence: Synthetic oligonucleotide
  source 1..50: mol_type = other DNA
atgacatagcctacctttacgcggggtaataggtgacgaccacagtatgg

SEQ ID NO: 16 - DNA, 50 bp, synthetic construct
  misc_feature 1..50: note = Description of Artificial Sequence: Synthetic oligonucleotide
  source 1..50: mol_type = other DNA
gtcgtgaggacagcttttgggacgaggcacccaggacatcaacaattcac

SEQ ID NO: 17 - DNA, 50 bp, synthetic construct
  misc_feature 1..50: note = Description of Artificial Sequence: Synthetic oligonucleotide
  source 1..50: mol_type = other DNA
tctaaatcaacccattatgccggatcggccggatcgcgggttcgagaagc

SEQ ID NO: 18 - DNA, 50 bp, synthetic construct
  misc_feature 1..50: note = Description of Artificial Sequence: Synthetic oligonucleotide
  source 1..50: mol_type = other DNA
acatcatcacagggaccataggcccgtctcttgatggaatatccgtgtcg

SEQ ID NO: 19 - DNA, 50 bp, synthetic construct
  misc_feature 1..50: note = Description of Artificial Sequence: Synthetic oligonucleotide
  source 1..50: mol_type = other DNA
gttcgctggttaaaacggtcacgcggctttgcttcagcaacacacaaggt

SEQ ID NO: 20 - DNA, 50 bp, synthetic construct
  misc_feature 1..50: note = Description of Artificial Sequence: Synthetic oligonucleotide
  source 1..50: mol_type = other DNA
tacctgcctaccgtggcatcacagccgtcgtaaggaactcgtggtaaaat

SEQ ID NO: 21 - DNA, 50 bp, synthetic construct
  misc_feature 1..50: note = Description of Artificial Sequence: Synthetic oligonucleotide
  source 1..50: mol_type = other DNA
ggcctcgatttctgcaaggtatcgcaccccggcccaggacccgtaaagcg

SEQ ID NO: 22 - DNA, 50 bp, synthetic construct
  misc_feature 1..50: note = Description of Artificial Sequence: Synthetic oligonucleotide
  source 1..50: mol_type = other DNA
actacgcacgtgatgccgtgaattaacgaactcgtcgacggcagagtcct

SEQ ID NO: 23 - DNA, 50 bp, synthetic construct
  misc_feature 1..50: note = Description of Artificial Sequence: Synthetic oligonucleotide
  source 1..50: mol_type = other DNA
cccacagaacggagaaggtcgaatgcaacagaacatagcgcgacggaggt

SEQ ID NO: 24 - DNA, 50 bp, synthetic construct
  misc_feature 1..50: note = Description of Artificial Sequence: Synthetic oligonucleotide
  source 1..50: mol_type = other DNA
aatgctctaaacgtaggcgatataggcggtaatacggatgctcctcttgt

SEQ ID NO: 25 - DNA, 50 bp, synthetic construct
  misc_feature 1..50: note = Description of Artificial Sequence: Synthetic oligonucleotide
  source 1..50: mol_type = other DNA
ctattacgccgtccaatgaccatataagccgacagctgtgtgggatttac

SEQ ID NO: 26 - DNA, 50 bp, synthetic construct
  misc_feature 1..50: note = Description of Artificial Sequence: Synthetic oligonucleotide
  source 1..50: mol_type = other DNA
tctgcgaactgatgcaaattgctatgcttgtaacctctatggctgtctgg

SEQ ID NO: 27 - DNA, 20 bp, synthetic construct
  misc_feature 1..20: note = Description of Artificial Sequence: Synthetic oligonucleotide
  source 1..20: mol_type = other DNA
gtaaaggtaggctatgtcat

SEQ ID NO: 28 - DNA, 30 bp, synthetic construct
  misc_feature 1..30: note = Description of Artificial Sequence: Synthetic oligonucleotide
  source 1..30: mol_type = other DNA
gtgcctcgtcccaaaagctgtcctcacgac

SEQ ID NO: 29 - DNA, 40 bp, synthetic construct
  misc_feature 1..40: note = Description of Artificial Sequence: Synthetic oligonucleotide
  source 1..40: mol_type = other DNA
gcttctcgaacccgcgatccggccgatccggcataatggg

SEQ ID NO: 30 - DNA, 50 bp, synthetic construct
  misc_feature 1..50: note = Description of Artificial Sequence: Synthetic oligonucleotide
  source 1..50: mol_type = other DNA
cgacacggatattccatcaagagacgggcctatggtccctgtgatgatgt

SEQ ID NO: 31 - DNA, 60 bp, synthetic construct
  misc_feature 1..60: note = Description of Artificial Sequence: Synthetic oligonucleotide
  source 1..60: mol_type = other DNA
attttaccacaccttgtgtgttgctgaagcaaagccgcgtgaccgttttaaccagcgaac

SEQ ID NO: 32 - DNA, 70 bp, synthetic construct
  misc_feature 1..70: note = Description of Artificial Sequence: Synthetic oligonucleotide
  source 1..70: mol_type = other DNA
ccattcgggcataatatgaactatacgcagcttatcccgggcccgtaacaaacaatttgcgtgaggtatg

SEQ ID NO: 33 - DNA, 80 bp, synthetic construct
  misc_feature 1..80: note = Description of Artificial Sequence: Synthetic oligonucleotide
  source 1..80: mol_type = other DNA
gtcccactcagagaattagcagccctggtctagcgagggatgccgcttagcgtcggttgaatttcgctgcactacagacg

SEQ ID NO: 34 - DNA, 90 bp, synthetic construct
  misc_feature 1..90: note = Description of Artificial Sequence: Synthetic oligonucleotide
  source 1..90: mol_type = other DNA
cgctttacgggtcctgggccggggtgcgataccttgcagaatctgcgcctcttggtggcgccccatcagtagtgtctacacgggcgctgt

SEQ ID NO: 35 - DNA, 100 bp, synthetic construct
  misc_feature 1..100: note = Description of Artificial Sequence: Synthetic polynucleotide
  source 1..100: mol_type = other DNA
gtaaatcccacacagctgtcggcttatatggtcattggacggcgtaatagacaagaggagcatccgtattaccgcctatatcgcctacgtttagagcatt

SEQ ID NO: 36 - DNA, 110 bp, synthetic construct
  misc_feature 1..110: note = Description of Artificial Sequence: Synthetic polynucleotide
  source 1..110: mol_type = other DNA
ggttcctaacaggtgattaccagtgcagttagccatttatcctcgtcaaaaagccacgttccagacagccatagaggttacaagcatagcaatttgcatcagttcgcaga

SEQ ID NO: 37 - DNA, 120 bp, synthetic construct
  misc_feature 1..120: note = Description of Artificial Sequence: Synthetic polynucleotide
  source 1..120: mol_type = other DNA
gacggccctagtctgcttctcgagacaatctgctagaactcggacgcctcgcactgtactgatgcatggtccgtaatcgaggtgaaaactacacggtatgacatcagcgataactggttt

SEQ ID NO: 38 - DNA, 33 bp, synthetic construct
  misc_feature 1..33: note = Description of Artificial Sequence: Synthetic oligonucleotide
  source 1..33: mol_type = other DNA
acactctttccctacacgacgctcttccgatct

SEQ ID NO: 39 - DNA, 34 bp, synthetic construct
  misc_feature 1..34: note = Description of Artificial Sequence: Synthetic oligonucleotide
  source 1..34: mol_type = other DNA
agatcggaagagcacacgtctgaactccagtcac

SEQ ID NO: 40 - DNA, 40 bp, synthetic construct
  misc_difference 1..7: note = a, c, t, g, unknown or other
  misc_feature 1..40: note = Description of Artificial Sequence: Synthetic oligonucleotide
  source 1..40: mol_type = other DNA
nnnnnnnagatcggaagagcgtcgtgtagggaaagagtgt

SEQ ID NO: 41 - DNA, 41 bp, synthetic construct
  misc_difference 35..41: note = a, c, t, g, unknown or other
  misc_feature 1..41: note = Description of Artificial Sequence: Synthetic oligonucleotide
  source 1..41: mol_type = other DNA
gtgactggagttcagacgtgtgctcttccgatctnnnnnnn